European Patent Application EP 4 209 215 A1, published July 12, 2023. Title: Treatment of Sandhoff disease. Applicant: Azafaros B.V. The sequence listing filed with the application follows.

SEQUENCE LISTING (3 sequences)

SEQ ID NO: 1 - DNA, 21 bp, Artificial Sequence
  Artificial Sequece
attttaaaattcaggcctcga

SEQ ID NO: 2 - DNA, 21 bp, Artificial Sequence
  Artifficial Sequence
catagcgttggctacccgtga

SEQ ID NO: 3 - DNA, 21 bp, Artificial Sequence
  Artificial Sequence
cattctgcagcggtgcacggc